European Patent Application EP 4 810 068 A1, published September 23, 2026. Title: 一种重组腺相关病毒药物组合物及其用途. Applicant: 成都弘基生物科技有限公司. The sequence listing filed with the application follows.

SEQUENCE LISTING (4 sequences)

SEQ ID NO: 1 - protein, 432 aa, synthetic construct
SDTGRPFVEMYSEIPEIIHMTEGRELVIPCRVTSPNITVTLKKFPLDTLIPDGKRIIWDSRKGFIISNATYKEIGLLTCEATVNGHLYKTNYLTHRQTNTIIDVVLSPSHGIELSVGEKLVLNCTARTELNVGIDFNWEYPSSKHQHKKLVNRDLKTQSGSEMKKFLSTLTIDGVTRSDQGLYTCAASSGLMTKKNSTFVRVHEKDKTHTCPPCPAPELLGGPSVFLFPPKPKDTLMISRTPEVTCVVVDVSHEDPEVKFNWYVDGVEVHNAKTKPREEQYNSTYRVVSVLTVLHQDWLNGKEYKCKVSNKALPAPIEKTISKAKGQPREPQVYTLPPSRDELTKNQVSLTCLVKGFYPSDIAVEWESNGQPENNYKTTPPVLDSDGSFFLYSKLTVDKSRWQQGNVFSCSVMHEALHNHYTQKSLSLSPGK

SEQ ID NO: 2 - DNA, 1459 bp, synthetic construct
  source 1..1459: mol_type = other DNA
atggtgtcctattgggatacaggagtgctgctgtgtgctctgctgagctgtctgctgctgacaggctcttcttcaggcaggtgagtatctcagggatccagacatggggatatgggaggtgcctctgatcccagggctcactgtgggtctctctgttcacagggacacaggcagaccctttgtggagatgtactctgaaatccctgagatcattcacatgacagaaggcagagaactggtgattccctgcagggttaccagcccaaacatcacagtgaccctgaagaagttccccctggacaccctgatccctgatggcaaaagaatcatctgggactctaggaaaggctttatcatctccaatgccacatacaaagagattggcctgctgacctgtgaggctactgtcaatggccacctgtacaaaacaaattacctgacccacagacagaccaacacaatcattgatgtggtgctgagcccatcccatggcattgagctgtctgtgggagaaaagctggtgctgaattgtacagctagaacagaacttaatgtgggcattgatttcaactgggagtaccctagctccaagcaccagcataaaaagctggtgaacagagacctgaagacccagtctggctctgagatgaaaaagttcttgagcaccctgaccattgatggagtgaccagatctgaccagggcctgtacacctgtgctgcctcctctgggctgatgacaaaaaagaacagcacctttgtgagagtgcatgagaaggataaaacccacacctgccctccttgtcctgctcctgagctgctggggggaccatctgtgttcctgttcccccccaagcccaaggataccctgatgatcagcagaaccccagaagtgacctgtgtggtggtggatgtgtcccatgaggacccagaggtgaaattcaactggtatgtggatggagtggaggtgcacaatgccaagaccaaaccaagagaggagcagtataactccacctacagggtggtgtctgtgctgactgtgctgcaccaggattggctgaatggcaaggagtacaagtgcaaggttagcaataaagctctgcctgcccccattgaaaagaccatttccaaagccaaagggcagccaagggagccccaggtgtacaccctgcccccatctagagatgagctgaccaagaaccaggtgagcctcacatgtctggtgaagggcttttacccttctgacattgctgtggagtgggaaagcaatggacagcctgagaataactataagaccacacccccagtgctggattctgatggcagttttttcctgtactctaagctgacagtggacaaatccagatggcagcagggcaatgtgttcagctgctctgtgatgcatgaggccctgcacaatcactatacacagaagagcctgagcctgagcccagggaagtga

SEQ ID NO: 3 - DNA, 3781 bp, synthetic construct
  source 1..3781: mol_type = other DNA
ctgcgcgctcgctcgctcactgaggccgcccgggcaaagcccgggcgtcgggcgacctttggtcgcccggcctcagtgagcgagcgagcgcgcagagagggagtggccaactccatcactaggggttccttgtagttaatgattaacccgccatgctacttatctaccagggtaatggggatcctctagaactatagctagtcgacattgattattgactagttattaatagtaatcaattacggggtcattagttcatagcccatatatggagttccgcgttacataacttacggtaaatggcccgcctggctgaccgcccaacgacccccgcccattgacgtcaataatgacgtatgttcccatagtaacgccaatagggactttccattgacgtcaatgggtggagtatttacggtaaactgcccacttggcagtacatcaagtgtatcatatgccaagtacgccccctattgacgtcaatgacggtaaatggcccgcctggcattatgcccagtacatgaccttatgggactttcctacttggcagtacatctacgtattagtcatcgctattaccatggtcgaggtgagccccacgttctgcttcactctccccatctcccccccctccccacccccaattttgtatttatttattttttaattattttgtgcagcgatgggggcggggggggggggggggcgcgcgccaggcggggcggggcggggcgaggggcggggcggggcgaggcggagaggtgcggcggcagccaatcagagcggcgcgctccgaaagtttccttttatggcgaggcggcggcggcggcggccctataaaaagcgaagcgcgcggcgggcggggagtcgctgcgacgctgccttcgccccgtgccccgctccgccgccgcctcgcgccgcccgccccggctctgactgaccgcgttactcccacaggtgagcgggcgggacggcccttctcctccgggctgtaattagcgcttggtttaatgacggcttgtttcttttctgtggctgcgtgaaagccttgaggggctccgggagggccctttgtgcggggggagcggctcggggggtgcgtgcgtgtgtgtgtgcgtggggagcgccgcgtgcggctccgcgctgcccggcggctgtgagcgctgcgggcgcggcgcggggctttgtgcgctccgcagtgtgcgcgaggggagcgcggccgggggcggtgccccgcggtgcggggggggctgcgaggggaacaaaggctgcgtgcggggtgtgtgcgtgggggggtgagcagggggtgtgggcgcgtcggtcgggctgcaaccccccctgcacccccctccccgagttgctgagcacggcccggcttcgggtgcggggctccgtacggggcgtggcgcggggctcgccgtgccgggcggggggtggcggcaggtgggggtgccgggcggggcggggccgcctcgggccggggagggctcgggggaggggcgcggcggcccccggagcgccggcggctgtcgaggcgcggcgagccgcagccattgccttttatggtaatcgtgcgagagggcgcagggacttcctttgtcccaaatctgtgcggagccgaaatctgggaggcgccgccgcaccccctctagcgggcgcggggcgaagcggtgcggcgccggcaggaaggaaatgggcggggagggccttcgtgcgtcgccgcgccgccgtccccttctccctctccagcctcggggctgtccgcggggggacggctgccttcgggggggacggggcagggcggggttcggcttctggcgtgtgaccggcggctctagagcctctgctaaccatgttcatgccttcttctttttcctacagctcctgggcaacgtgctggttattgtgctgtctcatcattttggcaaagaattcgccgccaccatggtgtcctattgggatacaggagtgctgctgtgtgctctgctgagctgtctgctgctgacaggctcttcttcaggcaggtgagtatctcagggatccagacatggggatatgggaggtgcctctgatcccagggctcactgtgggtctctctgttcacagggacacaggcagaccctttgtggagatgtactctgaaatccctgagatcattcacatgacagaaggcagagaactggtgattccctgcagggttaccagcccaaacatcacagtgaccctgaagaagttccccctggacaccctgatccctgatggcaaaagaatcatctgggactctaggaaaggctttatcatctccaatgccacatacaaagagattggcctgctgacctgtgaggctactgtcaatggccacctgtacaaaacaaattacctgacccacagacagaccaacacaatcattgatgtggtgctgagcccatcccatggcattgagctgtctgtgggagaaaagctggtgctgaattgtacagctagaacagaacttaatgtgggcattgatttcaactgggagtaccctagctccaagcaccagcataaaaagctggtgaacagagacctgaagacccagtctggctctgagatgaaaaagttcttgagcaccctgaccattgatggagtgaccagatctgaccagggcctgtacacctgtgctgcctcctctgggctgatgacaaaaaagaacagcacctttgtgagagtgcatgagaaggataaaacccacacctgccctccttgtcctgctcctgagctgctggggggaccatctgtgttcctgttcccccccaagcccaaggataccctgatgatcagcagaaccccagaagtgacctgtgtggtggtggatgtgtcccatgaggacccagaggtgaaattcaactggtatgtggatggagtggaggtgcacaatgccaagaccaaaccaagagaggagcagtataactccacctacagggtggtgtctgtgctgactgtgctgcaccaggattggctgaatggcaaggagtacaagtgcaaggttagcaataaagctctgcctgcccccattgaaaagaccatttccaaagccaaagggcagccaagggagccccaggtgtacaccctgcccccatctagagatgagctgaccaagaaccaggtgagcctcacatgtctggtgaagggcttttacccttctgacattgctgtggagtgggaaagcaatggacagcctgagaataactataagaccacacccccagtgctggattctgatggcagttttttcctgtactctaagctgacagtggacaaatccagatggcagcagggcaatgtgttcagctgctctgtgatgcatgaggccctgcacaatcactatacacagaagagcctgagcctgagcccagggaagtgactcgaggacggggtgaactacgcctgaggatccgatctttttccctctgccaaaaattatggggacatcatgaagccccttgagcatctgacttctggctaataaaggaaatttattttcattgcaatagtgtgttggaattttttgtgtctctcactcggaagcaattcgttgatctgaatttcgaccacccataatacccattaccctggtagataagtagcatggcgggttaatcattaactacaaggaacccctagtgatggagttggccactccctctctgcgcgctcgctcgctcactgaggccgggcgaccaaaggtcgcccgacgcccgggctttgcccgggcggcctcagtgagcgagcgagcgcgcag

SEQ ID NO: 4 - protein, 10 aa, synthetic construct
RGNQQNTARQ